European Patent Application EP 4 534 675 A1, published April 9, 2025. Title: A method for site-directed insterting an exogenous sequence in a genome. Applicant: Institute of Genetics and Developmental Biology, Chinese Academy of Sciences. Application CN. The sequence listing filed with the application follows.

SEQUENCE LISTING (103 sequences)

SEQ ID NO: 1 - protein, 1368 aa, synthetic construct [sequence omitted]

SEQ ID NO: 2 - protein, 1368 aa, synthetic construct
MDKKYSIGLDIGTNSVGWAVITDEYKVPSKKFKVLGNTDRHSIKKNLIGALLFDSGETAEATRLKRTARRRYTRRKNRICYLQEIFSNEMAKVDDSFFHRLEESFLVEEDKKHERHPIFGNIVDEVAYHEKYPTIYHLRKKLVDSTDKADLRLIYLALAHMIKFRGHFLIEGDLNPDNSDVDKLFIQLVQTYNQLFEENPINASGVDAKAILSARLSKSRRLENLIAQLPGEKKNGLFGNLIALSLGLTPNFKSNFDLAEDAKLQLSKDTYDDDLDNLLAQIGDQYADLFLAAKNLSDAILLSDILRVNTEITKAPLSASMIKRYDEHHQDLTLLKALVRQQLPEKYKEIFFDQSKNGYAGYIDGGASQEEFYKFIKPILEKMDGTEELLVKLNREDLLRKQRTFDNGSIPHQIHLGELHAILRRQEDFYPFLKDNREKIEKILTFRIPYYVGPLARGNSRFAWMTRKSEETITPWNFEEVVDKGASAQSFIERMTNFDKNLPNEKVLPKHSLLYEYFTVYNELTKVKYVTEGMRKPAFLSGEQKKAIVDLLFKTNRKVTVKQLKEDYFKKIECFDSVEISGVEDRFNASLGTYHDLLKIIKDKDFLDNEENEDILEDIVLTLTLFEDREMIEERLKTYAHLFDDKVMKQLKRRRYTGWGRLSRKLINGIRDKQSGKTILDFLKSDGFANRNFMQLIHDDSLTFKEDIQKAQVSGQGDSLHEHIANLAGSPAIKKGILQTVKVVDELVKVMGRHKPENIVIEMARENQTTQKGQKNSRERMKRIEEGIKELGSQILKEHPVENTQLQNEKLYLYYLQNGRDMYVDQELDINRLSDYDVDAIVPQSFLKDDSIDNKVLTRSDKNRGKSDNVPSEEVVKKMKNYWRQLLNAKLITQRKFDNLTKAERGGLSELDKAGFIKRQLVETRQITKHVAQILDSRMNTKYDENDKLIREVKVITLKSKLVSDFRKDFQFYKVREINNYHHAHDAYLNAVVGTALIKKYPKLESEFVYGDYKVYDVRKMIAKSEQEIGKATAKYFFYSNIMNFFKTEITLANGEIRKRPLIETNGETGEIVWDKGRDFATVRKVLSMPQVNIVKKTEVQTGGFSKESILPKRNSDKLIARKKDWDPKKYGGFDSPTVAYSVLVVAKVEKGKSKKLKSVKELLGITIMERSSFEKNPIDFLEAKGYKEVKKDLIIKLPKYSLFELENGRKRMLASAGELQKGNELALPSKYVNFLYLASHYEKLKGSPEDNEQKQLFVEQHKHYLDEIIEQISEFSKRVILADANLDKVLSAYNKHRDKPIREQAENIIHLFTLTNLGAPAAFKYFDTTIDRKRYTSTKEVLDATLIHQSITGLYETRIDLSQLGGD

SEQ ID NO: 3 - protein, 677 aa, synthetic construct
TLNIEDEYRLHETSKEPDVSLGSTWLSDFPQAWAETGGMGLAVRQAPLIIPLKATSTPVSIKQYPMSQEARLGIKPHIQRLLDQGILVPCQSPWNTPLLPVKKPGTNDYRPVQDLREVNKRVEDIHPTVPNPYNLLSGLPPSHQWYTVLDLKDAFFCLRLHPTSQPLFAFEWRDPEMGISGQLTWTRLPQGFKNSPTLFNEALHRDLADFRIQHPDLILLQYVDDLLLAATSELDCQQGTRALLQTLGNLGYRASAKKAQICQKQVKYLGYLLKEGQRWLTEARKETVMGQPTPKTPRQLREFLGKAGFCRLFIPGFAEMAAPLYPLTKPGTLFNWGPDQQKAYQEIKQALLTAPALGLPDLTKPFELFVDEKQGYAKGVLTQKLGPWRRPVAYLSKKLDPVAAGWPPCLRMVAAIAVLTKDAGKLTMGQPLVILAPHAVEALVKQPPDRWLSNARMTHYQALLLDTDRVQFGPVVALNPATLLPLPEEGLQHNCLDILAEAHGTRPDLTDQPLPDADHTWYTDGSSLLQEGQRKAGAAVTTETEVIWAKALPAGTSAQRAELIALTQALKMAEGKKLNVYTDSRYAFATAHIHGEIYRRRGWLTSEGKEIKNKDEILALLKALFLPKRLSIIHCPGHQKGHSAEARGNRMADQAARKAAITETPDTSTLLIENSSP

SEQ ID NO: 4 - protein, 129 aa, synthetic construct
DQQKAYQEIKQALLTAPALGLPDLTKPFELFVDEKQGYAKGVLTQKLGPWRRPVAYLSKKLDPVAAGWPPCLRMVAAIAVLTKDAGKLTMGQPLVILAPHAVEALVKQPPDRWLSNARMTHYQALLLDT

SEQ ID NO: 5 - protein, 157 aa, synthetic construct
PDADHTWYTDGSSLLQEGQRKAGAAVTTETEVIWAKALPAGTSAQRAELIALTQALKMAEGKKLNVYTDSRYAFATAHIHGEIYRRRGWLTSEGKEIKNKDEILALLKALFLPKRLSIIHCPGHQKGHSAEARGNRMADQAARKAAITETPDTSTLL

SEQ ID NO: 6 - protein, 56 aa, synthetic construct
ATVVSGQKQDRQGGERRRSQLDRDQCAYCKEKGHWAKDCPKKPRGPRGPRPQTSLL

SEQ ID NO: 7 - protein, 125 aa, synthetic construct
TLDDQGGQGQEPPPEPRITLKVGGQPVTFLVDTGAQHSVLTQNPGPLSDKSAWVQGATGGKRYRWTTDRKVHLATGKVTHSFLHVPDCPYPLLGRDLLTKLKAQIHFEGSGAQVMGPMGQPLQVL

SEQ ID NO: 8 - protein, 407 aa, synthetic construct
ENSSPYTSEHFHYTVTDIKDLTKLGAIYDKTKKYWVYQGKPVMPDQFTFELLDFLHQLTHLSFSKMKALLERSHSPYYMLNRDRTLKNITETCKACAQVNASKSAVKQGTRVRGHRPGTHWEIDFTEIKPGLYGYKYLLVFIDTFSGWIEAFPTKKETAKVVTKKLLEEIFPRFGMPQVLGTDNGPAFVSKVSQTVADLLGIDWKLHCAYRPQSSGQVERMNRTIKETLTKLTLATGSRDWVLLLPLALYRARNTPGPHGLTPYEILYGAPPPLVNFPDPDMTRVTNSPSLQAHLQALYLVQHEVWRPLAAAYQEQLDRPVVPHPYRVGDTVWVRRHQTKNLEPRWKGPYTVLLTTPTALKVDGIAAWIHAAHVKAADPGGGPSSRLTWRVQRSQNPLKIRLTREAP

SEQ ID NO: 9 - protein, 677 aa, synthetic construct
TLNIEDEYRLHETSKEPDVSLGSTWLSDFPQAWAETGGMGLAVRQAPLIIPLKATSTPVSIKQYPMSQEARLGIKPHIQRLLDQGILVPCQSPWNTPLLPVKKPGTNDYRPVQDLREVNKRVEDIHPTVPNPYNLLSGLPPSHQWYTVLDLKDAYFCLRLHPTSQPLFAFEWRDPEMGISGQLTWTRLPQGFKNSPTLFNEALHRDLADFRIQHPDLILLQYVDDLLLAATSELDCQQGTRALLQTLGNLGYRASAKKAQICQKQVKYLGYLLKEGQRWLTEARKETVMGQPTPKTPRQLREFLGKAGFCRLFIPGFAEMAAPLYPLTKPGTLFNWGPDQQKAYQEIKQALLTAPALGLPDLTKPFELFVDEKQGYAKGVLTQKLGPWRRPVAYLSKKLDPVAAGWPPCLRMVAAIAVLTKDAGKLTMGQPLVILAPHAVEALVKQPPDRWLSNARMTHYQALLLDTDRVQFGPVVALNPATLLPLPEEGLQHNCLDILAEAHGTRPDLTDQPLPDADHTWYTDGSSLLQEGQRKAGAAVTTETEVIWAKALPAGTSAQRAELIALTQALKMAEGKKLNVYTDSRYAFATAHIHGEIYRRRGWLTSEGKEIKNKDEILALLKALFLPKRLSIIHCPGHQKGHSAEARGNRMADQAARKAAITETPDTSTLLIENSSP

SEQ ID NO: 10 - protein, 677 aa, synthetic construct
TLNIEDEYRLHETSKEPDVSLGSTWLSDFPQAWAETGGMGLAVRQAPLIIPLKATSTPVSIKQYPMSQEARLGIKPHIQRLLDQGILVPCQSPWNTPLLPVKKPGTNDYRPVQDLREVNKRVEDIHPTVPNPYNLLSGLPPSHQWYTVLDLKDAVFCLRLHPTSQPLFAFEWRDPEMGISGQLTWTRLPQGFKNSPTLFNEALHRDLADFRIQHPDLILLQYVDDLLLAATSELDCQQGTRALLQTLGNLGYRASAKKAQICQKQVKYLGYLLKEGQRWLTEARKETVMGQPTPKTPRQLREFLGKAGFCRLFIPGFAEMAAPLYPLTKPGTLFNWGPDQQKAYQEIKQALLTAPALGLPDLTKPFELFVDEKQGYAKGVLTQKLGPWRRPVAYLSKKLDPVAAGWPPCLRMVAAIAVLTKDAGKLTMGQPLVILAPHAVEALVKQPPDRWLSNARMTHYQALLLDTDRVQFGPVVALNPATLLPLPEEGLQHNCLDILAEAHGTRPDLTDQPLPDADHTWYTDGSSLLQEGQRKAGAAVTTETEVIWAKALPAGTSAQRAELIALTQALKMAEGKKLNVYTDSRYAFATAHIHGEIYRRRGWLTSEGKEIKNKDEILALLKALFLPKRLSIIHCPGHQKGHSAEARGNRMADQAARKAAITETPDTSTLLIENSSP

SEQ ID NO: 11 - protein, 677 aa, synthetic construct
TLNIEDEYRLHETSKEPDVSLGSTWLSDFPQAWAETGGMGLAVRQAPLIIPLKATSTPVSIKQYPMSQEARLGIKPHIQRLLDQGILVPCQSPWNTPLLPVKKPGTNDYRPVQDLREVNKRVEDIHPTVPNPYNLLSGLPPSHQWYTVLDLKDAFYCLRLHPTSQPLFAFEWRDPEMGISGQLTWTRLPQGFKNSPTLFNEALHRDLADFRIQHPDLILLQYVDDLLLAATSELDCQQGTRALLQTLGNLGYRASAKKAQICQKQVKYLGYLLKEGQRWLTEARKETVMGQPTPKTPRQLREFLGKAGFCRLFIPGFAEMAAPLYPLTKPGTLFNWGPDQQKAYQEIKQALLTAPALGLPDLTKPFELFVDEKQGYAKGVLTQKLGPWRRPVAYLSKKLDPVAAGWPPCLRMVAAIAVLTKDAGKLTMGQPLVILAPHAVEALVKQPPDRWLSNARMTHYQALLLDTDRVQFGPVVALNPATLLPLPEEGLQHNCLDILAEAHGTRPDLTDQPLPDADHTWYTDGSSLLQEGQRKAGAAVTTETEVIWAKALPAGTSAQRAELIALTQALKMAEGKKLNVYTDSRYAFATAHIHGEIYRRRGWLTSEGKEIKNKDEILALLKALFLPKRLSIIHCPGHQKGHSAEARGNRMADQAARKAAITETPDTSTLLIENSSP

SEQ ID NO: 12 - protein, 677 aa, synthetic construct
TLNIEDEYRLHETSKEPDVSLGSTWLSDFPQAWAETGGMGLAVRQAPLIIPLKATSTPVSIKQYPMSQEARLGIKPHIQRLLDQGILVPCQSPWNTPLLPVKKPGTNDYRPVQDLREVNKRVEDIHPTVPNPYNLLSGLPPSHQWYTVLDLKDAFFCLRLHPTSQPLFAFEWRDPEMGISGQLTWTRLPQGFKNSPTLFNEALHRDLADFRIQHPDLILLQYVDDLLLAATSELDCQQGTRALLQTLGNLGYRASAKKAQICQKQVKYLGYLLKEGQRWLTEARKETVMGQPTPKTPRQLREFLGKAGFCRLFIPGFAEMAAPLYPLTKPGTLFNWGPDQQKAYQEIKQALLTAPALGLPDLTKPFELFVDEKQGYAKGVLTQKLGPWRRPVAYLSKKLDPVAAGWPPCLRMVAAIAVLTKDAGKLTMGQPLVILAPHAVEALVKQPPDRWLSNARMTHYQALLLDTDRVQFGPVVALNPATLLPLPEEGLQHNCLDILAEAHGTRPDLTDQPLPDADHTWYTNGSSLLQEGQRKAGAAVTTETEVIWAKALPAGTSAQRAELIALTQALKMAEGKKLNVYTDSRYAFATAHIHGEIYRRRGWLTSEGKEIKNKDEILALLKALFLPKRLSIIHCPGHQKGHSAEARGNRMADQAARKAAITETPDTSTLLIENSSP

SEQ ID NO: 13 - protein, 677 aa, synthetic construct
TLNIEDEYRLHETSKEPDVSLGSTWLSDFPQAWAETGGMGLAVRQAPLIIPLKATSTPVSIKQYPMSQEARLGIKPHIQRLLDQGILVPCQSPWNTPLLPVKKPGTNDYRPVQDLREVNKRVEDIHPTVPNPYNLLSGLPPSHQWYTVLDLKDAYFCLRLHPTSQPLFAFEWRDPEMGISGQLTWTRLPQGFKNSPTLFCEALHRDLADFRIQHPDLILLQYVDDLLLAATSELDCQQGTRALLQTLGNLGYRASAKKAQICQKQVKYLGYLLKEGQRWLTEARKETVMGQPTPKTPRQLREFLGKAGFCRLFIPGFAEMAAPLYPLTKPGTLFNWGPDQQKAYQEIKQALLTAPALGLPDLTKPFELFVDEKQGYAKGVLTQKLGPWRRPVAYLSKKLDPVAAGWPPCLRMVAAIAVLTKDAGKLTMGQPLVILAPHAVEALVKQPPDRWLSNARMTHYQALLLDTDRVQFGPVVALNPATLLPLPEEGLQHNCLDILAEAHGTRPDLTDQPLPDADHTWYTDGSSLLQEGQRKAGAAVTTETEVIWAKALPAGTSAQRAELIALTQALKMAEGKKLNVYTDSRYAFATAHIHGEIYRRRGWLTSEGKEIKNKDEILALLKALFLPKRLSIIHCPGHQKGHSAEARGNRMADQAARKAAITETPDTSTLLIENSSP

SEQ ID NO: 14 - protein, 514 aa, synthetic construct
TLNIEDEYRLHETSKEPDVSLGSTWLSDFPQAWAETGGMGLAVRQAPLIIPLKATSTPVSIKQYPMSQEARLGIKPHIQRLLDQGILVPCQSPWNTPLLPVKKPGTNDYRPVQDLREVNKRVEDIHPTVPNPYNLLSGLPPSHQWYTVLDLKDAFFCLRLHPTSQPLFAFEWRDPEMGISGQLTWTRLPQGFKNSPTLFNEALHRDLADFRIQHPDLILLQYVDDLLLAATSELDCQQGTRALLQTLGNLGYRASAKKAQICQKQVKYLGYLLKEGQRWLTEARKETVMGQPTPKTPRQLREFLGKAGFCRLFIPGFAEMAAPLYPLTKPGTLFNWGPDQQKAYQEIKQALLTAPALGLPDLTKPFELFVDEKQGYAKGVLTQKLGPWRRPVAYLSKKLDPVAAGWPPCLRMVAAIAVLTKDAGKLTMGQPLVILAPHAVEALVKQPPDRWLSNARMTHYQALLLDTDRVQFGPVVALNPATLLPLPEEGLQHNCLDILAEAHGTRPDLTDQPL

SEQ ID NO: 15 - protein, 338 aa, synthetic construct
TLNIEDEYRLHETSKEPDVSLGSTWLSDFPQAWAETGGMGLAVRQAPLIIPLKATSTPVSIKQYPMSQEARLGIKPHIQRLLDQGILVPCQSPWNTPLLPVKKPGTNDYRPVQDLREVNKRVEDIHPTVPNPYNLLSGLPPSHQWYTVLDLKDAFFCLRLHPTSQPLFAFEWRDPEMGISGQLTWTRLPQGFKNSPTLFNEALHRDLADFRIQHPDLILLQYVDDLLLAATSELDCQQGTRALLQTLGNLGYRASAKKAQICQKQVKYLGYLLKEGQRWLTEARKETVMGQPTPKTPRQLREFLGKAGFCRLFIPGFAEMAAPLYPLTKPGTLFNWGP

SEQ ID NO: 16 - protein, 32 aa, synthetic construct
SGGSSGGSSGSETPGTSESATPESSGGSSGGS

SEQ ID NO: 17 - RNA, 76 nt, synthetic construct
  source 1..76: mol_type = other RNA
gttttagagctagaaatagcaagttaaaataaggctagtccgttatcaacttgaaaaagtggcaccgagtcggtgc

SEQ ID NO: 18 - protein, 2108 aa, synthetic construct
MPKKKRKVDKKYSIGLDIGTNSVGWAVITDEYKVPSKKFKVLGNTDRHSIKKNLIGALLFDSGETAEATRLKRTARRRYTRRKNRICYLQEIFSNEMAKVDDSFFHRLEESFLVEEDKKHERHPIFGNIVDEVAYHEKYPTIYHLRKKLVDSTDKADLRLIYLALAHMIKFRGHFLIEGDLNPDNSDVDKLFIQLVQTYNQLFEENPINASGVDAKAILSARLSKSRRLENLIAQLPGEKKNGLFGNLIALSLGLTPNFKSNFDLAEDAKLQLSKDTYDDDLDNLLAQIGDQYADLFLAAKNLSDAILLSDILRVNTEITKAPLSASMIKRYDEHHQDLTLLKALVRQQLPEKYKEIFFDQSKNGYAGYIDGGASQEEFYKFIKPILEKMDGTEELLVKLNREDLLRKQRTFDNGSIPHQIHLGELHAILRRQEDFYPFLKDNREKIEKILTFRIPYYVGPLARGNSRFAWMTRKSEETITPWNFEEVVDKGASAQSFIERMTNFDKNLPNEKVLPKHSLLYEYFTVYNELTKVKYVTEGMRKPAFLSGEQKKAIVDLLFKTNRKVTVKQLKEDYFKKIECFDSVEISGVEDRFNASLGTYHDLLKIIKDKDFLDNEENEDILEDIVLTLTLFEDREMIEERLKTYAHLFDDKVMKQLKRRRYTGWGRLSRKLINGIRDKQSGKTILDFLKSDGFANRNFMQLIHDDSLTFKEDIQKAQVSGQGDSLHEHIANLAGSPAIKKGILQTVKVVDELVKVMGRHKPENIVIEMARENQTTQKGQKNSRERMKRIEEGIKELGSQILKEHPVENTQLQNEKLYLYYLQNGRDMYVDQELDINRLSDYDVDAIVPQSFLKDDSIDNKVLTRSDKNRGKSDNVPSEEVVKKMKNYWRQLLNAKLITQRKFDNLTKAERGGLSELDKAGFIKRQLVETRQITKHVAQILDSRMNTKYDENDKLIREVKVITLKSKLVSDFRKDFQFYKVREINNYHHAHDAYLNAVVGTALIKKYPKLESEFVYGDYKVYDVRKMIAKSEQEIGKATAKYFFYSNIMNFFKTEITLANGEIRKRPLIETNGETGEIVWDKGRDFATVRKVLSMPQVNIVKKTEVQTGGFSKESILPKRNSDKLIARKKDWDPKKYGGFDSPTVAYSVLVVAKVEKGKSKKLKSVKELLGITIMERSSFEKNPIDFLEAKGYKEVKKDLIIKLPKYSLFELENGRKRMLASAGELQKGNELALPSKYVNFLYLASHYEKLKGSPEDNEQKQLFVEQHKHYLDEIIEQISEFSKRVILADANLDKVLSAYNKHRDKPIREQAENIIHLFTLTNLGAPAAFKYFDTTIDRKRYTSTKEVLDATLIHQSITGLYETRIDLSQLGGDEFPKKKRKVELSGGSSGGSSGSETPGTSESATPESSGGSSGGSRPTLNIEDEYRLHETSKEPDVSLGSTWLSDFPQAWAETGGMGLAVRQAPLIIPLKATSTPVSIKQYPMSQEARLGIKPHIQRLLDQGILVPCQSPWNTPLLPVKKPGTNDYRPVQDLREVNKRVEDIHPTVPNPYNLLSGLPPSHQWYTVLDLKDAFFCLRLHPTSQPLFAFEWRDPEMGISGQLTWTRLPQGFKNSPTLFNEALHRDLADFRIQHPDLILLQYVDDLLLAATSELDCQQGTRALLQTLGNLGYRASAKKAQICQKQVKYLGYLLKEGQRWLTEARKETVMGQPTPKTPRQLREFLGKAGFCRLFIPGFAEMAAPLYPLTKPGTLFNWGPDQQKAYQEIKQALLTAPALGLPDLTKPFELFVDEKQGYAKGVLTQKLGPWRRPVAYLSKKLDPVAAGWPPCLRMVAAIAVLTKDAGKLTMGQPLVILAPHAVEALVKQPPDRWLSNARMTHYQALLLDTDRVQFGPVVALNPATLLPLPEEGLQHNCLDILAEAHGTRPDLTDQPLPDADHTWYTDGSSLLQEGQRKAGAAVTTETEVIWAKALPAGTSAQRAELIALTQALKMAEGKKLNVYTDSRYAFATAHIHGEIYRRRGWLTSEGKEIKNKDEILALLKALFLPKRLSIIHCPGHQKGHSAEARGNRMADQAARKAAITETPDTSTLLIENSSPSGGSPKKKRKV

SEQ ID NO: 19 - protein, 2017 aa, synthetic construct
MPKKKRKVDKKYSIGLDIGTNSVGWAVITDEYKVPSKKFKVLGNTDRHSIKKNLIGALLFDSGETAEATRLKRTARRRYTRRKNRICYLQEIFSNEMAKVDDSFFHRLEESFLVEEDKKHERHPIFGNIVDEVAYHEKYPTIYHLRKKLVDSTDKADLRLIYLALAHMIKFRGHFLIEGDLNPDNSDVDKLFIQLVQTYNQLFEENPINASGVDAKAILSARLSKSRRLENLIAQLPGEKKNGLFGNLIALSLGLTPNFKSNFDLAEDAKLQLSKDTYDDDLDNLLAQIGDQYADLFLAAKNLSDAILLSDILRVNTEITKAPLSASMIKRYDEHHQDLTLLKALVRQQLPEKYKEIFFDQSKNGYAGYIDGGASQEEFYKFIKPILEKMDGTEELLVKLNREDLLRKQRTFDNGSIPHQIHLGELHAILRRQEDFYPFLKDNREKIEKILTFRIPYYVGPLARGNSRFAWMTRKSEETITPWNFEEVVDKGASAQSFIERMTNFDKNLPNEKVLPKHSLLYEYFTVYNELTKVKYVTEGMRKPAFLSGEQKKAIVDLLFKTNRKVTVKQLKEDYFKKIECFDSVEISGVEDRFNASLGTYHDLLKIIKDKDFLDNEENEDILEDIVLTLTLFEDREMIEERLKTYAHLFDDKVMKQLKRRRYTGWGRLSRKLINGIRDKQSGKTILDFLKSDGFANRNFMQLIHDDSLTFKEDIQKAQVSGQGDSLHEHIANLAGSPAIKKGILQTVKVVDELVKVMGRHKPENIVIEMARENQTTQKGQKNSRERMKRIEEGIKELGSQILKEHPVENTQLQNEKLYLYYLQNGRDMYVDQELDINRLSDYDVDAIVPQSFLKDDSIDNKVLTRSDKNRGKSDNVPSEEVVKKMKNYWRQLLNAKLITQRKFDNLTKAERGGLSELDKAGFIKRQLVETRQITKHVAQILDSRMNTKYDENDKLIREVKVITLKSKLVSDFRKDFQFYKVREINNYHHAHDAYLNAVVGTALIKKYPKLESEFVYGDYKVYDVRKMIAKSEQEIGKATAKYFFYSNIMNFFKTEITLANGEIRKRPLIETNGETGEIVWDKGRDFATVRKVLSMPQVNIVKKTEVQTGGFSKESILPKRNSDKLIARKKDWDPKKYGGFDSPTVAYSVLVVAKVEKGKSKKLKSVKELLGITIMERSSFEKNPIDFLEAKGYKEVKKDLIIKLPKYSLFELENGRKRMLASAGELQKGNELALPSKYVNFLYLASHYEKLKGSPEDNEQKQLFVEQHKHYLDEIIEQISEFSKRVILADANLDKVLSAYNKHRDKPIREQAENIIHLFTLTNLGAPAAFKYFDTTIDRKRYTSTKEVLDATLIHQSITGLYETRIDLSQLGGDEFSGSETPGTSESATPESATVVSGQKQDRQGGERRRSQLDRDQCAYCKEKGHWAKDCPKKPRGPRGPRPQTSLLPKKKRKVELSGGSSGGSSGSETPGTSESATPESSGGSSGGSRPTLNIEDEYRLHETSKEPDVSLGSTWLSDFPQAWAETGGMGLAVRQAPLIIPLKATSTPVSIKQYPMSQEARLGIKPHIQRLLDQGILVPCQSPWNTPLLPVKKPGTNDYRPVQDLREVNKRVEDIHPTVPNPYNLLSGLPPSHQWYTVLDLKDAFFCLRLHPTSQPLFAFEWRDPEMGISGQLTWTRLPQGFKNSPTLFNEALHRDLADFRIQHPDLILLQYVDDLLLAATSELDCQQGTRALLQTLGNLGYRASAKKAQICQKQVKYLGYLLKEGQRWLTEARKETVMGQPTPKTPRQLREFLGKAGFCRLFIPGFAEMAAPLYPLTKPGTLFNWGPDQQKAYQEIKQALLTAPALGLPDLTKPFELFVDEKQGYAKGVLTQKLGPWRRPVAYLSKKLDPVAAGWPPCLRMVAAIAVLTKDAGKLTMGQPLVILAPHAVEALVKQPPDRWLSNARMTHYQALLLDTDRVQFGPVVALNPATLLPLPEEGLQHNCLDILAEAHGTRPDLTDQPLSGGSPKKKRKV

SEQ ID NO: 20 - DNA, 37 bp, synthetic construct
  source 1..37: mol_type = other DNA
cgcggttctatctagttacgcgttaaaccaactagaa

SEQ ID NO: 21 - DNA, 994 bp, synthetic construct
  source 1..994: mol_type = other DNA
atggagtcaaagattcaaatagaggacctaacagaactcgccgtaaagactggcgaacagttcatacagagtctcttacgactcaatgacaagaagaaaatcttcgtcaacatggtggagcacgacacacttgtctactccaaaaatatcaaagatacagtctcagaagaccaaagggcaattgagacttttcaacaaagggtaatatccggaaacctcctcggattccattgcccagctatctgtcactttattgtgaagatagtggaaaaggaaggtggctcctacaaatgccatcattgcgataaaggaaaggccatcgttgaagatgcctctgccgacagtggtcccaaagatggacccccacccacgaggagcatcgtggaaaaagaagacgttccaaccacgtcttcaaagcaagtggattgatgtgattggcagacatactgtcccacaaatgaagatggaatctgtaaaagaaaacgcgtgaaataatgcgtctgacaaaggttaggtcggctgcctttaatcaataccaaagtggtccctaccacgatggaaaaactgtgcagtcggtttggctttttctgacgaacaaataagattcgtggccgacaggtgggggtccaccatgtgaaggcatcttcagactccaataatggagcaatgacgtaagggcttacgaaataagtaagggtagtttgggaaatgtccactcacccgtcagtctataaatacttagcccctccctcattgttaagggagcaaaatctcagagagatagtcctagagagagaaagagagcaagtagcctagaagtagtcaaggcggcgaagtattcaggcacgtggccaggaagaagaaaagccaagacgacgaaaacaggtaagagctaagcatctagataagttgaaaacaatcttcaaaagtcccacatcgcttagataagaaaacgaagctgagtttatatacagctagagtcgaagtagtgatt

SEQ ID NO: 22 - protein, 605 aa, synthetic construct
MDTYAGAYDRQSRERENSSAASPATQRSANEDKAADLQREVERDGGRFRFVGHFSEAPGTSAFGTAERPEFERILNECRAGRLNMIIVYDVSRFSRLKVMDAIPIVSELLALGVTIVSTQEGVFRQGNVMDLIHLIMRLDASHKESSLKSAKILDTKNLQRELGGYVGGKAPYGFELVSETKEITRNGRMVNVVINKLAHSTTPLTGPFEFEPDVIRWWWREIKTHKHLPFKPGSQAAIHPGSITGLCKRMDADAVPTRGETIGKKTASSAWDPATVMRILRDPRIAGFAAEVIYKKKPDGTPTTKIEGYRIQRDPITLRPVELDCGPIIEPAEWYELQAWLDGRGRGKGLSRGQAILSAMDKLYCECGAVMTSKRGEESIKDSYRCRRRKVVDPSAPGQHEGTCNVSMAALDKFVAERIFNKIRHAEGDEETLALLWEAARRFGKLTEAPEKSGERANLVAERADALNALEELYEDRAAGAYDGPVGRKHFRKQQAALTLRQQGAEERLAELEAAEAPKLPLDQWFPEDADADPTGPKSWWGRASVDDKRVFVGLFVDKIVVTKSTTGRGQGTPIEKRASITWAKPPTDDDEDDAQDGTEDVAA

SEQ ID NO: 23 - protein, 502 aa, synthetic construct
MRALVVIRLSRVTDATTSPERQLESCQQLCAQRGWDVVGVAEDLDVSGAVDPFDRKRRPNLARWLAFEEQPFDVIVAYRVDRLTRSIRHLQQLVHWAEDHKKLVVSATEAHFDTTTPFAAVVIALMGTVAQMELEAIKERNRSAAHFNIRAGKYRGSLPPWGYLPTRVDGEWRLVPDPVQRERILEVYHRVVDNHEPLHLVAHDLNRRGVLSPKDYFAQLQGREPQGREWSATALKRSMISEAMLGYATLNGKTVRDDDGAPLVRAEPILTREQLEALRAELVKTSRAKPAVSTPSLLLRVLFCAVCGEPAYKFAGGGRKHPRYRCRSMGFPKHCGNGTVAMAEWDAFCEEQVLDLLGDAERLEKVWVAGSDSAVELAEVNAELVDLTSLIGSPAYRAGSPQREALDARIAALAARQEELEGLEARPSGWEWRETGQRFGDWWREQDTAAKNTWLRSMNVRLTFDVRGGLTRTIDFGDLQEYEQHLRLGSVVERLHTGMSEF

SEQ ID NO: 24 - protein, 342 aa, synthetic construct
SNLLTVHQNLPALPVDATSDEVRKNLMDMFRDRQAFSEHTWKMLLSVCRSWAAWCKLNNRKWFPAEPEDVRDYLLYLQARGLAVKTIQQHLGQLNMLHRRSGLPRPSDSNAVSLVMRRIRKENVDAGERAKQALAFERTDFDQVRSLMENSDRCQDIRNLAFLGIAYNTLLRIAEIARIRVKDISRTDGGRMLIHIGRTKTLVSTAGVEKALSLGVTKLVERWISVSGVADDPNNYLFCRVRKNGVAAPSATSQLSTRALEGIFEATHRLIYGAKDDSGQRYLAWSGHSARVGAARDMARAGVSIPEIMQAGGWTNVNIVMNYIRNLDSETGAMVRLLEDGD

SEQ ID NO: 25 - protein, 423 aa, synthetic construct
MPQFDILCKTPPKVLVRQFVERFERPSGEKIALCAAELTYLCWMITHNGTAIKRATFMSYNTIISNSLSFDIVNKSLQFKYKTQKATILEASLKKLIPAWEFTIIPYYGQKHQSDITDIVSSLQLQFESSEEADKGNSHSKKMLKALLSEGESIWEITEKILNSFEYTSRFTKTKTLYQFLFLATFINCGRFSDIKNVDPKSFKLVQNKYLGVIIQCLVTETKTSVSRHIYFFSARGRIDPLVYLDEFLRNSEPVLKRVNRTGNSSSNKQEYQLLKDNLVRSYNKALKKNAPYSIFAIKNGPKSHIGRHLMTSFLSMKGLTELTNVVGNWSDKRASAVARTTYTHQITAIPDHYFALVSRYYAYDPISKEMIALKDETNPIEEWQHIEQLKGSAEGSIRYPAWNGIISQEVLDYLSSYINRRI

SEQ ID NO: 26 - DNA, 34 bp, synthetic construct
  source 1..34: mol_type = other DNA
ataacttcgtatagcatacattatacgaagttat

SEQ ID NO: 27 - DNA, 34 bp, synthetic construct
  source 1..34: mol_type = other DNA
ataacttcgtatagcatacattatacgaacggta

SEQ ID NO: 28 - DNA, 34 bp, synthetic construct
  source 1..34: mol_type = other DNA
taccgttcgtatagcatacattatacgaagttat

SEQ ID NO: 29 - DNA, 34 bp, synthetic construct
  source 1..34: mol_type = other DNA
ataacttcgtataggatactttatacgaagttat

SEQ ID NO: 30 - DNA, 48 bp, synthetic construct
  source 1..48: mol_type = other DNA
gaagttcctattccgaagttcctattctctagaaagtataggaacttc

SEQ ID NO: 31 - DNA, 48 bp, synthetic construct
  source 1..48: mol_type = other DNA
gaagttcctattccgaagttcctattcttcaaaaagtataggaacttc

SEQ ID NO: 32 - DNA, 48 bp, synthetic construct
  source 1..48: mol_type = other DNA
ggaggtcttatttcgaagttcctattctctagaaagtataggaacttc

SEQ ID NO: 33 - DNA, 48 bp, synthetic construct
  source 1..48: mol_type = other DNA
gaagttcctattccggaggtcttattttctagaaagtataggaacttc

SEQ ID NO: 34 - DNA, 48 bp, synthetic construct
  source 1..48: mol_type = other DNA
ggaggtcttatttcgaagttcctattctctagaaagtataagacctcc

SEQ ID NO: 35 - DNA, 34 bp, synthetic construct
  source 1..34: mol_type = other DNA
gaagttcctattctctagaaagtataggaacttc

SEQ ID NO: 36 - DNA, 34 bp, synthetic construct
  source 1..34: mol_type = other DNA
ggaggtcttattttctagaaagtataggaacttc

SEQ ID NO: 37 - DNA, 34 bp, synthetic construct
  source 1..34: mol_type = other DNA
gaagttcctattctctagaaagtataagacctcc

SEQ ID NO: 38 - DNA, 50 bp, synthetic construct
  source 1..50: mol_type = other DNA
gtagtgccccaactggggtaacctttgagttctctcagttgggggcgtag

SEQ ID NO: 39 - DNA, 50 bp, synthetic construct
  source 1..50: mol_type = other DNA
cggtgcgggtgccagggcgtgcccttgggctccccgggcgcgtactccac

SEQ ID NO: 40 - DNA, 48 bp, synthetic construct
  source 1..48: mol_type = other DNA
ggtttgtctggtcaaccaccgcggtctcagtggtgtacggtacaaacc

SEQ ID NO: 41 - DNA, 46 bp, synthetic construct
  source 1..46: mol_type = other DNA
ggccggcttgtcgacgacggcggtctccgtcgtcaggatcatccgg

SEQ ID NO: 42 - protein, 1368 aa, synthetic construct
KDKKYSIGLDIGTNSVGWAVITDEYKVPSKKFKVLGNTDRHSIKKNLIGALLFDSGETAEATRLKRTARRRYTRRKNRICYLQEIFSNEMAKVDDSFFHRLEESFLVEEDKKHERHPIFGNIVDEVAYHEKYPTIYHLRKKLVDSTDKADLRLIYLALAHMIKFRGHFLIEGDLNPDNSDVDKLFIQLVQTYNQLFEENPINASGVDAKAILSARLSKSRRLENLIAQLPGEKKNGLFGNLIALSLGLTPNFKSNFDLAEDAKLQLSKDTYDDDLDNLLAQIGDQYADLFLAAKNLSDAILLSDILRVNTEITKAPLSASMIKRYDEHHQDLTLLKALVRQQLPEKYKEIFFDQSKNGYAGYIDGGASQEEFYKFIKPILEKMDGTEELLVKLNREDLLRKQRTFDNGSIPHQIHLGELHAILRRQEDFYPFLKDNREKIEKILTFRIPYYVGPLARGNSRFAWMTRKSEETITPWNFEEVVDKGASAQSFIERMTNFDKNLPNEKVLPKHSLLYEYFTVYNELTKVKYVTEGMRKPAFLSGEQKKAIVDLLFKTNRKVTVKQLKEDYFKKIECFDSVEISGVEDRFNASLGTYHDLLKIIKDKDFLDNEENEDILEDIVLTLTLFEDREMIEERLKTYAHLFDDKVMKQLKRRRYTGWGRLSRKLINGIRDKQSGKTILDFLKSDGFANRNFMQLIHDDSLTFKEDIQKAQVSGQGDSLHEHIANLAGSPAIKKGILQTVKVVDELVKVMGRHKPENIVIEMARENQTTQKGQKNSRERMKRIEEGIKELGSQILKEHPVENTQLQNEKLYLYYLQNGRDMYVDQELDINRLSDYDVDAIVPQSFLKDDSIDNKVLTRSDKNRGKSDNVPSEEVVKKMKNYWRQLLNAKLITQRKFDNLTKAERGGLSELDKAGFIKRQLVETRQITKHVAQILDSRMNTKYDENDKLIREVKVITLKSKLVSDFRKDFQFYKVREINNYHHAHDAYLNAVVGTALIKKYPKLESEFVYGDYKVYDVRKMIAKSEQEIGKATAKYFFYSNIMNFFKTEITLANGEIRKRPLIETNGETGEIVWDKGRDFATVRKVLSMPQVNIVKKTEVQTGGFSKESILPKRNSDKLIARKKDWDPKKYGGFLWPTVAYSVLVVAKVEKGKSKKLKSVKELLGITIMERSSFEKNPIDFLEAKGYKEVKKDLIIKLPKYSLFELENGRKRMLASAKQLQKGNELALPSKYVNFLYLASHYEKLKGSPEDNEQKQLFVEQHKHYLDEIIEQISEFSKRVILADANLDKVLSAYNKHRDKPIREQAENIIHLFTLTNLGAPAAFKYFDTTIDRKQYRSTKEVLDATLIHQSITGLYETRIDLSQLGGD

SEQ ID NO: 43 - protein, 1383 aa, synthetic construct
DKKYSIGLDIGTNSVGWAVITDEYKVPSKKFKVLGNTDRHSIKKNLIGALLFDSGETAERTRLKRTARRRYTRRKNRICYLQEIFSNEMAKVDDSFFHRLEESFLVEEDKKHERHPIFGNIVDEVAYHEKYPTIYHLRKKLVDSTDKADLRLIYLALAHMIKFRGHFLIEGDLNPDNSDVDKLFIQLVQTYNQLFEENPINASGVDAKAILSARLSKSRRLENLIAQLPGEKKNGLFGNLIALSLGLTPNFKSNFDLAEDAKLQLSKDTYDDDLDNLLAQIGDQYADLFLAAKNLSDAILLSDILRVNTEITKAPLSASMIKRYDEHHQDLTLLKALVRQQLPEKYKEIFFDQSKNGYAGYIDGGASQEEFYKFIKPILEKMDGTEELLVKLNREDLLRKQRTFDNGSIPHQIHLGELHAILRRQEDFYPFLKDNREKIEKILTFRIPYYVGPLARGNSRFAWMTRKSEETITPWNFEEVVDKGASAQSFIERMTNFDKNLPNEKVLPKHSLLYEYFTVYNELTKVKYVTEGMRKPAFLSGEQKKAIVDLLFKTNRKVTVKQLKEDYFKKIECFDSVEISGVEDRFNASLGTYHDLLKIIKDKDFLDNEENEDILEDIVLTLTLFEDREMIEERLKTYAHLFDDKVMKQLKRRRYTGWGRLSRKLINGIRDKQSGKTILDFLKSDGFANRNFMQLIHDDSLTFKEDIQKAQVSGQGDSLHEHIANLAGSPAIKKGILQTVKVVDELVKVMGRHKPENIVIEMARENQTTQKGQKNSRERMKRIEEGIKELGSQILKEHPVENTQLQNEKLYLYYLQNGRDMYVDQELDINRLSDYDVDAIVPQSFLKDDSIDNKVLTRSDKNRGKSDNVPSEEVVKKMKNYWRQLLNAKLITQRKFDNLTKAERGGLSELDKAGFIKRQLVETRQITKHVAQILDSRMNTKYDENDKLIREVKVITLKSKLVSDFRKDFQFYKVREINNYHHAHDAYLNAVVGTALIKKYPKLESEFVYGDYKVYDVRKMIAKSEQEIGKATAKYFFYSNIMNFFKTEITLANGEIRKRPLIETNGETGEIVWDKGRDFATVRKVLSMPQVNIVKKTEVQTGGFSKESIRPKRNSDKLIARKKDWDPKKYGGFLWPTVAYSVLVVAKVEKGKSKKLKSVKELLGITIMERSSFEKNPIDFLEAKGYKEVKKDLIIKLPKYSLFELENGRKRMLASAKQLQKGNELALPSKYVNFLYLASHYEKLKGSPEDNEQKQLFVEQHKHYLDEIIEQISEFSKRVILADANLDKVLSAYNKHRDKPIREQAENIIHLFTLTRLGAPRAFKYFDTTIDPKQYRSTKEVLDATLIHQSITGLYETRIDLSQLGGDKRPAATKKAGQAKKKK

SEQ ID NO: 44 - protein, 116 aa, synthetic construct
ASNFTQFVLVDNGGTGDVTVAPSNFANGIAEWISSNSRSQAYKVTCSVRQSSAQNRKYTIKVEVPKGAWRSYLNMELTIPIFATNSDCELIVKAMQGLLKDGNPIPSAIAANSGIY

SEQ ID NO: 45 - DNA, 67 bp, synthetic construct
  source 1..67: mol_type = other DNA
gggagcacatgaggatcacccatgtgccacgagcgacatgaggatcacccatgtcgctcgtgttccc

SEQ ID NO: 46 - protein, 2414 aa, synthetic construct
MPKKKRKVSGGSPKKKRKVSGGSSNLLTVHQNLPALPVDATSDEVRKNLMDMFRDRQAFSEHTWKMLLSVCRSWAAWCKLNNRKWFPAEPEDVRDYLLYLQARGLAVKTIQQHLGQLNMLHRRSGLPRPSDSNAVSLVMRRIRKENVDAGERAKQALAFERTDFDQVRSLMENSDRCQDIRNLAFLGIAYNTLLRIAEIARIRVKDISRTDGGRMLIHIGRTKTLVSTAGVEKALSLGVTKLVERWISVSGVADDPNNYLFCRVRKNGVAAPSATSQLSTRALEGIFEATHRLIYGAKDDSGQRYLAWSGHSARVGAARDMARAGVSIPEIMQAGGWTNVNIVMNYIRNLDSETGAMVRLLEDGDSGGSSGGSSGSETPGTSESATPESSGGSSGGSMPKKKRKVDKKYSIGLDIGTNSVGWAVITDEYKVPSKKFKVLGNTDRHSIKKNLIGALLFDSGETAEATRLKRTARRRYTRRKNRICYLQEIFSNEMAKVDDSFFHRLEESFLVEEDKKHERHPIFGNIVDEVAYHEKYPTIYHLRKKLVDSTDKADLRLIYLALAHMIKFRGHFLIEGDLNPDNSDVDKLFIQLVQTYNQLFEENPINASGVDAKAILSARLSKSRRLENLIAQLPGEKKNGLFGNLIALSLGLTPNFKSNFDLAEDAKLQLSKDTYDDDLDNLLAQIGDQYADLFLAAKNLSDAILLSDILRVNTEITKAPLSASMIKRYDEHHQDLTLLKALVRQQLPEKYKEIFFDQSKNGYAGYIDGGASQEEFYKFIKPILEKMDGTEELLVKLNREDLLRKQRTFDNGSIPHQIHLGELHAILRRQEDFYPFLKDNREKIEKILTFRIPYYVGPLARGNSRFAWMTRKSEETITPWNFEEVVDKGASAQSFIERMTNFDKNLPNEKVLPKHSLLYEYFTVYNELTKVKYVTEGMRKPAFLSGEQKKAIVDLLFKTNRKVTVKQLKEDYFKKIECFDSVEISGVEDRFNASLGTYHDLLKIIKDKDFLDNEENEDILEDIVLTLTLFEDREMIEERLKTYAHLFDDKVMKQLKRRRYTGWGRLSRKLINGIRDKQSGKTILDFLKSDGFANRNFMQLIHDDSLTFKEDIQKAQVSGQGDSLHEHIANLAGSPAIKKGILQTVKVVDELVKVMGRHKPENIVIEMARENQTTQKGQKNSRERMKRIEEGIKELGSQILKEHPVENTQLQNEKLYLYYLQNGRDMYVDQELDINRLSDYDVDAIVPQSFLKDDSIDNKVLTRSDKNRGKSDNVPSEEVVKKMKNYWRQLLNAKLITQRKFDNLTKAERGGLSELDKAGFIKRQLVETRQITKHVAQILDSRMNTKYDENDKLIREVKVITLKSKLVSDFRKDFQFYKVREINNYHHAHDAYLNAVVGTALIKKYPKLESEFVYGDYKVYDVRKMIAKSEQEIGKATAKYFFYSNIMNFFKTEITLANGEIRKRPLIETNGETGEIVWDKGRDFATVRKVLSMPQVNIVKKTEVQTGGFSKESILPKRNSDKLIARKKDWDPKKYGGFDSPTVAYSVLVVAKVEKGKSKKLKSVKELLGITIMERSSFEKNPIDFLEAKGYKEVKKDLIIKLPKYSLFELENGRKRMLASAGELQKGNELALPSKYVNFLYLASHYEKLKGSPEDNEQKQLFVEQHKHYLDEIIEQISEFSKRVILADANLDKVLSAYNKHRDKPIREQAENIIHLFTLTNLGAPAAFKYFDTTIDRKRYTSTKEVLDATLIHQSITGLYETRIDLSQLGGDEFSGSETPGTSESATPESATVVSGQKQDRQGGERRRSQLDRDQCAYCKEKGHWAKDCPKKPRGPRGPRPQTSLLPKKKRKVELSGGSSGGSSGSETPGTSESATPESSGGSSGGSRPTLNIEDEYRLHETSKEPDVSLGSTWLSDFPQAWAETGGMGLAVRQAPLIIPLKATSTPVSIKQYPMSQEARLGIKPHIQRLLDQGILVPCQSPWNTPLLPVKKPGTNDYRPVQDLREVNKRVEDIHPTVPNPYNLLSGLPPSHQWYTVLDLKDAFFCLRLHPTSQPLFAFEWRDPEMGISGQLTWTRLPQGFKNSPTLFNEALHRDLADFRIQHPDLILLQYVDDLLLAATSELDCQQGTRALLQTLGNLGYRASAKKAQICQKQVKYLGYLLKEGQRWLTEARKETVMGQPTPKTPRQLREFLGKAGFCRLFIPGFAEMAAPLYPLTKPGTLFNWGPDQQKAYQEIKQALLTAPALGLPDLTKPFELFVDEKQGYAKGVLTQKLGPWRRPVAYLSKKLDPVAAGWPPCLRMVAAIAVLTKDAGKLTMGQPLVILAPHAVEALVKQPPDRWLSNARMTHYQALLLDTDRVQFGPVVALNPATLLPLPEEGLQHNCLDILAEAHGTRPDLTDQPLSGGSPKKKRKV

SEQ ID NO: 47 - protein, 2496 aa, synthetic construct
MPKKKRKVSGGSPKKKRKVSGGSSMPQFDILCKTPPKVLVRQFVERFERPSGEKIALCAAELTYLCWMITHNGTAIKRATFMSYNTIISNSLSFDIVNKSLQFKYKTQKATILEASLKKLIPAWEFTIIPYYGQKHQSDITDIVSSLQLQFESSEEADKGNSHSKKMLKALLSEGESIWEITEKILNSFEYTSRFTKTKTLYQFLFLATFINCGRFSDIKNVDPKSFKLVQNKYLGVIIQCLVTETKTSVSRHIYFFSARGRIDPLVYLDEFLRNSEPVLKRVNRTGNSSSNKQEYQLLKDNLVRSYNKALKKNAPYSIFAIKNGPKSHIGRHLMTSFLSMKGLTELTNVVGNWSDKRASAVARTTYTHQITAIPDHYFALVSRYYAYDPISKEMIALKDETNPIEEWQHIEQLKGSAEGSIRYPAWNGIISQEVLDYLSSYINRRISGGSSGGSSGSETPGTSESATPESSGGSSGGSMPKKKRKVDKKYSIGLDIGTNSVGWAVITDEYKVPSKKFKVLGNTDRHSIKKNLIGALLFDSGETAEATRLKRTARRRYTRRKNRICYLQEIFSNEMAKVDDSFFHRLEESFLVEEDKKHERHPIFGNIVDEVAYHEKYPTIYHLRKKLVDSTDKADLRLIYLALAHMIKFRGHFLIEGDLNPDNSDVDKLFIQLVQTYNQLFEENPINASGVDAKAILSARLSKSRRLENLIAQLPGEKKNGLFGNLIALSLGLTPNFKSNFDLAEDAKLQLSKDTYDDDLDNLLAQIGDQYADLFLAAKNLSDAILLSDILRVNTEITKAPLSASMIKRYDEHHQDLTLLKALVRQQLPEKYKEIFFDQSKNGYAGYIDGGASQEEFYKFIKPILEKMDGTEELLVKLNREDLLRKQRTFDNGSIPHQIHLGELHAILRRQEDFYPFLKDNREKIEKILTFRIPYYVGPLARGNSRFAWMTRKSEETITPWNFEEVVDKGASAQSFIERMTNFDKNLPNEKVLPKHSLLYEYFTVYNELTKVKYVTEGMRKPAFLSGEQKKAIVDLLFKTNRKVTVKQLKEDYFKKIECFDSVEISGVEDRFNASLGTYHDLLKIIKDKDFLDNEENEDILEDIVLTLTLFEDREMIEERLKTYAHLFDDKVMKQLKRRRYTGWGRLSRKLINGIRDKQSGKTILDFLKSDGFANRNFMQLIHDDSLTFKEDIQKAQVSGQGDSLHEHIANLAGSPAIKKGILQTVKVVDELVKVMGRHKPENIVIEMARENQTTQKGQKNSRERMKRIEEGIKELGSQILKEHPVENTQLQNEKLYLYYLQNGRDMYVDQELDINRLSDYDVDAIVPQSFLKDDSIDNKVLTRSDKNRGKSDNVPSEEVVKKMKNYWRQLLNAKLITQRKFDNLTKAERGGLSELDKAGFIKRQLVETRQITKHVAQILDSRMNTKYDENDKLIREVKVITLKSKLVSDFRKDFQFYKVREINNYHHAHDAYLNAVVGTALIKKYPKLESEFVYGDYKVYDVRKMIAKSEQEIGKATAKYFFYSNIMNFFKTEITLANGEIRKRPLIETNGETGEIVWDKGRDFATVRKVLSMPQVNIVKKTEVQTGGFSKESILPKRNSDKLIARKKDWDPKKYGGFDSPTVAYSVLVVAKVEKGKSKKLKSVKELLGITIMERSSFEKNPIDFLEAKGYKEVKKDLIIKLPKYSLFELENGRKRMLASAGELQKGNELALPSKYVNFLYLASHYEKLKGSPEDNEQKQLFVEQHKHYLDEIIEQISEFSKRVILADANLDKVLSAYNKHRDKPIREQAENIIHLFTLTNLGAPAAFKYFDTTIDRKRYTSTKEVLDATLIHQSITGLYETRIDLSQLGGDEFSGSETPGTSESATPESATVVSGQKQDRQGGERRRSQLDRDQCAYCKEKGHWAKDCPKKPRGPRGPRPQTSLLPKKKRKVELSGGSSGGSSGSETPGTSESATPESSGGSSGGSRPTLNIEDEYRLHETSKEPDVSLGSTWLSDFPQAWAETGGMGLAVRQAPLIIPLKATSTPVSIKQYPMSQEARLGIKPHIQRLLDQGILVPCQSPWNTPLLPVKKPGTNDYRPVQDLREVNKRVEDIHPTVPNPYNLLSGLPPSHQWYTVLDLKDAFFCLRLHPTSQPLFAFEWRDPEMGISGQLTWTRLPQGFKNSPTLFNEALHRDLADFRIQHPDLILLQYVDDLLLAATSELDCQQGTRALLQTLGNLGYRASAKKAQICQKQVKYLGYLLKEGQRWLTEARKETVMGQPTPKTPRQLREFLGKAGFCRLFIPGFAEMAAPLYPLTKPGTLFNWGPDQQKAYQEIKQALLTAPALGLPDLTKPFELFVDEKQGYAKGVLTQKLGPWRRPVAYLSKKLDPVAAGWPPCLRMVAAIAVLTKDAGKLTMGQPLVILAPHAVEALVKQPPDRWLSNARMTHYQALLLDTDRVQFGPVVALNPATLLPLPEEGLQHNCLDILAEAHGTRPDLTDQPLSGGSPKKKRKV

SEQ ID NO: 48 - protein, 2418 aa, synthetic construct
MPKKKRKVDKKYSIGLDIGTNSVGWAVITDEYKVPSKKFKVLGNTDRHSIKKNLIGALLFDSGETAEATRLKRTARRRYTRRKNRICYLQEIFSNEMAKVDDSFFHRLEESFLVEEDKKHERHPIFGNIVDEVAYHEKYPTIYHLRKKLVDSTDKADLRLIYLALAHMIKFRGHFLIEGDLNPDNSDVDKLFIQLVQTYNQLFEENPINASGVDAKAILSARLSKSRRLENLIAQLPGEKKNGLFGNLIALSLGLTPNFKSNFDLAEDAKLQLSKDTYDDDLDNLLAQIGDQYADLFLAAKNLSDAILLSDILRVNTEITKAPLSASMIKRYDEHHQDLTLLKALVRQQLPEKYKEIFFDQSKNGYAGYIDGGASQEEFYKFIKPILEKMDGTEELLVKLNREDLLRKQRTFDNGSIPHQIHLGELHAILRRQEDFYPFLKDNREKIEKILTFRIPYYVGPLARGNSRFAWMTRKSEETITPWNFEEVVDKGASAQSFIERMTNFDKNLPNEKVLPKHSLLYEYFTVYNELTKVKYVTEGMRKPAFLSGEQKKAIVDLLFKTNRKVTVKQLKEDYFKKIECFDSVEISGVEDRFNASLGTYHDLLKIIKDKDFLDNEENEDILEDIVLTLTLFEDREMIEERLKTYAHLFDDKVMKQLKRRRYTGWGRLSRKLINGIRDKQSGKTILDFLKSDGFANRNFMQLIHDDSLTFKEDIQKAQVSGQGDSLHEHIANLAGSPAIKKGILQTVKVVDELVKVMGRHKPENIVIEMARENQTTQKGQKNSRERMKRIEEGIKELGSQILKEHPVENTQLQNEKLYLYYLQNGRDMYVDQELDINRLSDYDVDAIVPQSFLKDDSIDNKVLTRSDKNRGKSDNVPSEEVVKKMKNYWRQLLNAKLITQRKFDNLTKAERGGLSELDKAGFIKRQLVETRQITKHVAQILDSRMNTKYDENDKLIREVKVITLKSKLVSDFRKDFQFYKVREINNYHHAHDAYLNAVVGTALIKKYPKLESEFVYGDYKVYDVRKMIAKSEQEIGKATAKYFFYSNIMNFFKTEITLANGEIRKRPLIETNGETGEIVWDKGRDFATVRKVLSMPQVNIVKKTEVQTGGFSKESILPKRNSDKLIARKKDWDPKKYGGFDSPTVAYSVLVVAKVEKGKSKKLKSVKELLGITIMERSSFEKNPIDFLEAKGYKEVKKDLIIKLPKYSLFELENGRKRMLASAGELQKGNELALPSKYVNFLYLASHYEKLKGSPEDNEQKQLFVEQHKHYLDEIIEQISEFSKRVILADANLDKVLSAYNKHRDKPIREQAENIIHLFTLTNLGAPAAFKYFDTTIDRKRYTSTKEVLDATLIHQSITGLYETRIDLSQLGGDEFSGSETPGTSESATPESATVVSGQKQDRQGGERRRSQLDRDQCAYCKEKGHWAKDCPKKPRGPRGPRPQTSLLPKKKRKVELSGGSSGGSSGSETPGTSESATPESSGGSSGGSRPTLNIEDEYRLHETSKEPDVSLGSTWLSDFPQAWAETGGMGLAVRQAPLIIPLKATSTPVSIKQYPMSQEARLGIKPHIQRLLDQGILVPCQSPWNTPLLPVKKPGTNDYRPVQDLREVNKRVEDIHPTVPNPYNLLSGLPPSHQWYTVLDLKDAFFCLRLHPTSQPLFAFEWRDPEMGISGQLTWTRLPQGFKNSPTLFNEALHRDLADFRIQHPDLILLQYVDDLLLAATSELDCQQGTRALLQTLGNLGYRASAKKAQICQKQVKYLGYLLKEGQRWLTEARKETVMGQPTPKTPRQLREFLGKAGFCRLFIPGFAEMAAPLYPLTKPGTLFNWGPDQQKAYQEIKQALLTAPALGLPDLTKPFELFVDEKQGYAKGVLTQKLGPWRRPVAYLSKKLDPVAAGWPPCLRMVAAIAVLTKDAGKLTMGQPLVILAPHAVEALVKQPPDRWLSNARMTHYQALLLDTDRVQFGPVVALNPATLLPLPEEGLQHNCLDILAEAHGTRPDLTDQPLSGGSPKKKRKVSGGSSGGSSGSETPGTSESATPESSGGSSGGSPKKKRKVSGGSSNLLTVHQNLPALPVDATSDEVRKNLMDMFRDRQAFSEHTWKMLLSVCRSWAAWCKLNNRKWFPAEPEDVRDYLLYLQARGLAVKTIQQHLGQLNMLHRRSGLPRPSDSNAVSLVMRRIRKENVDAGERAKQALAFERTDFDQVRSLMENSDRCQDIRNLAFLGIAYNTLLRIAEIARIRVKDISRTDGGRMLIHIGRTKTLVSTAGVEKALSLGVTKLVERWISVSGVADDPNNYLFCRVRKNGVAAPSATSQLSTRALEGIFEATHRLIYGAKDDSGQRYLAWSGHSARVGAARDMARAGVSIPEIMQAGGWTNVNIVMNYIRNLDSETGAMVRLLEDGDKRPAATKKAGQAKKKK

SEQ ID NO: 49 - protein, 2500 aa, synthetic construct
MPKKKRKVDKKYSIGLDIGTNSVGWAVITDEYKVPSKKFKVLGNTDRHSIKKNLIGALLFDSGETAEATRLKRTARRRYTRRKNRICYLQEIFSNEMAKVDDSFFHRLEESFLVEEDKKHERHPIFGNIVDEVAYHEKYPTIYHLRKKLVDSTDKADLRLIYLALAHMIKFRGHFLIEGDLNPDNSDVDKLFIQLVQTYNQLFEENPINASGVDAKAILSARLSKSRRLENLIAQLPGEKKNGLFGNLIALSLGLTPNFKSNFDLAEDAKLQLSKDTYDDDLDNLLAQIGDQYADLFLAAKNLSDAILLSDILRVNTEITKAPLSASMIKRYDEHHQDLTLLKALVRQQLPEKYKEIFFDQSKNGYAGYIDGGASQEEFYKFIKPILEKMDGTEELLVKLNREDLLRKQRTFDNGSIPHQIHLGELHAILRRQEDFYPFLKDNREKIEKILTFRIPYYVGPLARGNSRFAWMTRKSEETITPWNFEEVVDKGASAQSFIERMTNFDKNLPNEKVLPKHSLLYEYFTVYNELTKVKYVTEGMRKPAFLSGEQKKAIVDLLFKTNRKVTVKQLKEDYFKKIECFDSVEISGVEDRFNASLGTYHDLLKIIKDKDFLDNEENEDILEDIVLTLTLFEDREMIEERLKTYAHLFDDKVMKQLKRRRYTGWGRLSRKLINGIRDKQSGKTILDFLKSDGFANRNFMQLIHDDSLTFKEDIQKAQVSGQGDSLHEHIANLAGSPAIKKGILQTVKVVDELVKVMGRHKPENIVIEMARENQTTQKGQKNSRERMKRIEEGIKELGSQILKEHPVENTQLQNEKLYLYYLQNGRDMYVDQELDINRLSDYDVDAIVPQSFLKDDSIDNKVLTRSDKNRGKSDNVPSEEVVKKMKNYWRQLLNAKLITQRKFDNLTKAERGGLSELDKAGFIKRQLVETRQITKHVAQILDSRMNTKYDENDKLIREVKVITLKSKLVSDFRKDFQFYKVREINNYHHAHDAYLNAVVGTALIKKYPKLESEFVYGDYKVYDVRKMIAKSEQEIGKATAKYFFYSNIMNFFKTEITLANGEIRKRPLIETNGETGEIVWDKGRDFATVRKVLSMPQVNIVKKTEVQTGGFSKESILPKRNSDKLIARKKDWDPKKYGGFDSPTVAYSVLVVAKVEKGKSKKLKSVKELLGITIMERSSFEKNPIDFLEAKGYKEVKKDLIIKLPKYSLFELENGRKRMLASAGELQKGNELALPSKYVNFLYLASHYEKLKGSPEDNEQKQLFVEQHKHYLDEIIEQISEFSKRVILADANLDKVLSAYNKHRDKPIREQAENIIHLFTLTNLGAPAAFKYFDTTIDRKRYTSTKEVLDATLIHQSITGLYETRIDLSQLGGDEFSGSETPGTSESATPESATVVSGQKQDRQGGERRRSQLDRDQCAYCKEKGHWAKDCPKKPRGPRGPRPQTSLLPKKKRKVELSGGSSGGSSGSETPGTSESATPESSGGSSGGSRPTLNIEDEYRLHETSKEPDVSLGSTWLSDFPQAWAETGGMGLAVRQAPLIIPLKATSTPVSIKQYPMSQEARLGIKPHIQRLLDQGILVPCQSPWNTPLLPVKKPGTNDYRPVQDLREVNKRVEDIHPTVPNPYNLLSGLPPSHQWYTVLDLKDAFFCLRLHPTSQPLFAFEWRDPEMGISGQLTWTRLPQGFKNSPTLFNEALHRDLADFRIQHPDLILLQYVDDLLLAATSELDCQQGTRALLQTLGNLGYRASAKKAQICQKQVKYLGYLLKEGQRWLTEARKETVMGQPTPKTPRQLREFLGKAGFCRLFIPGFAEMAAPLYPLTKPGTLFNWGPDQQKAYQEIKQALLTAPALGLPDLTKPFELFVDEKQGYAKGVLTQKLGPWRRPVAYLSKKLDPVAAGWPPCLRMVAAIAVLTKDAGKLTMGQPLVILAPHAVEALVKQPPDRWLSNARMTHYQALLLDTDRVQFGPVVALNPATLLPLPEEGLQHNCLDILAEAHGTRPDLTDQPLSGGSPKKKRKVSGGSSGGSSGSETPGTSESATPESSGGSSGGSPKKKRKVSGGSSMPQFDILCKTPPKVLVRQFVERFERPSGEKIALCAAELTYLCWMITHNGTAIKRATFMSYNTIISNSLSFDIVNKSLQFKYKTQKATILEASLKKLIPAWEFTIIPYYGQKHQSDITDIVSSLQLQFESSEEADKGNSHSKKMLKALLSEGESIWEITEKILNSFEYTSRFTKTKTLYQFLFLATFINCGRFSDIKNVDPKSFKLVQNKYLGVIIQCLVTETKTSVSRHIYFFSARGRIDPLVYLDEFLRNSEPVLKRVNRTGNSSSNKQEYQLLKDNLVRSYNKALKKNAPYSIFAIKNGPKSHIGRHLMTSFLSMKGLTELTNVVGNWSDKRASAVARTTYTHQITAIPDHYFALVSRYYAYDPISKEMIALKDETNPIEEWQHIEQLKGSAEGSIRYPAWNGIISQEVLDYLSSYINRRIKRPAATKKAGQAKKKK

SEQ ID NO: 50 - protein, 474 aa, synthetic construct
MSEFSELVRILPLDQVAEIKRILSRGDPIPLQRLASLLTMVILTVNMSKKRKSSPIKLSTFTKYRRNVAKSLYYDMSSKTVFFEYHLKNTQDLQEGLEQAIAPYNFVVKVHKKPIDWQKQLSSVHERKAGHRSILSNNVGAEISKLAETKDSTWSFIERTMDLIEARTRQPTTRVAYRFLLQLTFMNCCRANDLKNADPSTFQIIADPHLGRILRAFVPETKTSIERFIYFFPCKGRCDPLLALDSYLLWVGPVPKTQTTDEETQYDYQLLQDTLLISYDRFIAKESKENIFKIPNGPKAHLGRHLMASYLGNNSLKSEATLYGNWSVERQEGVSKMADSRYMHTVKKSPPSYLFAFLSGYYKKSNQGEYVLAETLYNPLDYDKTLPITTNEKLICRRYGKNAKVIPKDALLYLYTYAQQKRKQLADPNEQNRLFSSESPAHPFLTPQSTGSSTPLTWTAPKTLSTGLMTPGEE

SEQ ID NO: 51 - protein, 447 aa, synthetic construct
MSTFAEAAHLTPHQCANEINEILESDTFNINAKEIRNKLASLFSILTMQSLSIRREMKINTYRSYKSAIGKSLSFDKDDKIIKFTVRLRKTESLQKDIESALPSYKVVVSPFKNQEVSLFDRYEETHKYDASMVGLQFTNILSKEKDIWKIVSRIACFFDQSCVTTTKRAEYRLLLLGAVGNCCRYSDLKNLDPRTFEIYNNSFLGPIVRATVTETKSRTERYVNFYPVNGDCDLLISLYDYLRVCSPIEKTVSSNRPTNQTHQFLPESLARTFSRFLTQHVDEPVFKIWNGPKSHFGRHLMATFLSRSEKGKYVSSLGNWAGDREIQSAVARSHYSHGSVTVDDRVFAFISGFYKEAPLGSEIYVLKDPSNKPLSREELLEEEGNSLGSPPLSPPSSPRLVAQSFSAHPSLQLFEQWHGIISDEVLQFIAEYRRKHELRSQRTVVA

SEQ ID NO: 52 - protein, 490 aa, synthetic construct
MQLTKDTEISTINRQMSDFSELSQILPLHQISKIKDILENENPLPKEKLASHLTMIILMANLASQKRKDVPVKRSTFLKYQRSISKTLQYDSSTKTVSFEYHLKDPSKLIKGLEDVVSPYRFVVGVHEKPDDVMSHLSAVHMRKEAGRKRDLGNKINDEITKIAETQETIWGFVGKTMDLIEARTTRPTTKAAYNLLLQATFMNCCRADDLKNTDIKTFEVIPDKHLGRMLRAFVPETKTGTRFVYFFPCKGRCDPLLALDSYLQWTDPIPKTRTTDEDARYDYQLLRNSLLGSYDGFISKQSDESIFKIPNGPKAHLGRHVTASYLSNNEMDKEATLYGNWSAAREEGVSRVAKARYMHTIEKSPPSYLFAFLSGFYNITAERACELVDPNSNPCEQDKNIPMISDIETLMARYGKNAEIIPMDVLVFLSSYARFKNNEGKEYKLQARSSRGVPDFPDNGRTALYNALTAAHVKRRKISIVVGRSIDTS

SEQ ID NO: 53 - DNA, 36 bp, synthetic construct
  source 1..36: mol_type = other DNA
gagtttcattaaggaataactaattcaatgaaactc

SEQ ID NO: 54 - DNA, 61 bp, synthetic construct
  source 1..61: mol_type = other DNA
aaacgatatcagacatttgtctgataatgcttcattatcagacaaatgtctgatatcgttt

SEQ ID NO: 55 - DNA, 31 bp, synthetic construct
  source 1..31: mol_type = other DNA
ttgatgaaagaataacgtattctttcatcaa

SEQ ID NO: 56 - protein, 342 aa, synthetic construct
MSELIISGSSGGFLRNIGKEYQEAAENFMRFMNDQGAYAPNTLRDLRLVFHSWARWCHARQLAWFPISPEMAREYFLQLHDADLASTTIDKHYAMLNMLLSHCGLPPLSDDKSVSLAMRRIRREAATEKGERTGQAIPLRWDDLKLLDVLLSRSERLVDLRNRAFLFVAYNTLMRMSEISRIRVGDLDQTGDTVTLHISHTKTITTAAGLDKVLSRRTTAVLNDWLDVSGLREHPDAVLFPPIHRSNKARITTTPLTAPAMEKIFSDAWVLLNKRDATPNKGRYRTWTGHSARVGAAIDMAEKQVSMVEIMQEGTWKKPETLMRYLRRGGVSVGANSRLMDS

SEQ ID NO: 57 - DNA, 32 bp, synthetic construct
  source 1..32: mol_type = other DNA
taactttaaataatgccaattatttaaagtta

SEQ ID NO: 58 - DNA, 32 bp, synthetic construct
  source 1..32: mol_type = other DNA
taactttaaataatgtccattatttaaagtta

SEQ ID NO: 59 - DNA, 97 bp, synthetic construct
  source 1..97: mol_type = other DNA
gatcctgtgcaatttgaaaggaaccctgacgagattccgtgggctgaataacttcgtatagcatacattatacgaagttattcgaggtcattcatat

SEQ ID NO: 60 - DNA, 90 bp, synthetic construct
  source 1..90: mol_type = other DNA
ataccttcaagtgagcagcagccttctccttgtcagtgaagacactaccgttcgtataatgtatgctatacgaacggtaggtctacctac

SEQ ID NO: 61 - DNA, 97 bp, synthetic construct
  source 1..97: mol_type = other DNA
gatcctgtgcaatttgaaaggaaccctgacgagattccgtgggctgagggtgggcttggctttgttttcggtctccgcccccccgggcgtttttatg

SEQ ID NO: 62 - DNA, 87 bp, synthetic construct
  source 1..87: mol_type = other DNA
cagtgaagacaccggtggactccacgacatactcagcaccagccgggtgggcgggacctcttctacctacaaaaaagctccgcacga

SEQ ID NO: 63 - DNA, 29 bp, synthetic construct
  source 1..29: mol_type = other DNA
cgtggaactgatgtttgaaaggtggtata

SEQ ID NO: 64 - DNA, 76 bp, synthetic construct
  source 1..76: mol_type = other DNA
cgtggaactgatgtttatggctgggcttggccttgaattcgagctcggtaccctcgatcagttaaaaggtggtata

SEQ ID NO: 65 - DNA, 75 bp, synthetic construct
  source 1..75: mol_type = other DNA
cgtggaactgatgtttgctgggcttggccttgaattcgagctcggtaccctcgaggtcagttaaaaggtggtata

SEQ ID NO: 66 - DNA, 46 bp, synthetic construct
  source 1..46: mol_type = other DNA
cgtggaactgatgtttcagtacggaaaaagagttgaaggtggtata

SEQ ID NO: 67 - DNA, 70 bp, synthetic construct
  source 1..70: mol_type = other DNA
cgtggaactgatgtttgagggagaggcggtggctcgctgcgctcggtcgttcaagttaaaaggtggtata

SEQ ID NO: 68 - DNA, 73 bp, synthetic construct
  source 1..73: mol_type = other DNA
cgtggaactgatgttttgcgtttctgggtgagtcgagctcggtaccctcgaggtccagttaaaaggtggtata

SEQ ID NO: 69 - DNA, 67 bp, synthetic construct
  source 1..67: mol_type = other DNA
cgtggaactgatgttttggtcgttcgctccaagcctcgaggtcattcgaggtctaaaaggtggtata

SEQ ID NO: 70 - DNA, 74 bp, synthetic construct
  source 1..74: mol_type = other DNA
cgtggaactgatgtttgagttttcgttccactgacttaattcgagctcggtaccccgagttaaaaggtggtata

SEQ ID NO: 71 - DNA, 74 bp, synthetic construct
  source 1..74: mol_type = other DNA
cgtggaactgatgttttgaggtaagattacctggtcgaattcgagctcggtaccctcagttaaaaggtggtata

SEQ ID NO: 72 - DNA, 27 bp, synthetic construct
  source 1..27: mol_type = other DNA
cgtggaaaatccaaataaggtggtata

SEQ ID NO: 73 - DNA, 79 bp, synthetic construct
  source 1..79: mol_type = other DNA
cttttcatgatttgtgacaaatgcagcgaagaggtaccggccagccggctggtgctgagtatgtcgtggagtccaccgg

SEQ ID NO: 74 - DNA, 79 bp, synthetic construct
  source 1..79: mol_type = other DNA
cttttcatgatttgtgacaaatgcagcctagaagaggtaccggccagcctggtgctgagtatgtcgtggagtccaccgg

SEQ ID NO: 75 - DNA, 74 bp, synthetic construct
  source 1..74: mol_type = other DNA
cctttcatgatttgtgacaaatgcgaagaggtatctgcgttagccggtgctgagtatgtcgtggagtccaccgg

SEQ ID NO: 76 - DNA, 79 bp, synthetic construct
  source 1..79: mol_type = other DNA
cttttcacgatttgtgacaaatgcagcgaagaggtaccggccagccggctggtgctgagtgtgtcgtggagtccaccgg

SEQ ID NO: 77 - DNA, 72 bp, synthetic construct
  source 1..72: mol_type = other DNA
cttttcatgatttgtgacaaatggaagaggtacagaccccgttggtgctgagtatgtcgtggagtccaccgg

SEQ ID NO: 78 - DNA, 79 bp, synthetic construct; identical to SEQ ID NO: 76
  source 1..79: mol_type = other DNA

SEQ ID NO: 79 - DNA, 75 bp, synthetic construct
  source 1..75: mol_type = other DNA
cttttcatgatttgtgacaaatgcgaagaggtaccagctcggggctggtgctgagtatgtcgtggagtccaccgg

SEQ ID NO: 80 - DNA, 75 bp, synthetic construct
  source 1..75: mol_type = other DNA
cttttcatgatttgtggcaaatgcgaagaggtaccccagcctggctggtgctgagtatgtcgtggagtccaccgg

SEQ ID NO: 81 - DNA, 79 bp, synthetic construct
  source 1..79: mol_type = other DNA
cttttcatgatttgtgacaaatgcagcgaagaggtaccggccagtcggctggtgctgagtatgtcgtggagtccaccgg

SEQ ID NO: 82 - DNA, 79 bp, synthetic construct
  source 1..79: mol_type = other DNA
cttttcatgatttgtgacaaatgcatcaaagaggtaccggccagccggctggcgctgagtatgtcgaggagtccaccgg

SEQ ID NO: 83 - DNA, 49 bp, synthetic construct
  source 1..49: mol_type = other DNA
gaagcatctgtctgtcccccgtataaccgtatagcatacattatacgaa

SEQ ID NO: 84 - DNA, 56 bp, synthetic construct
  source 1..56: mol_type = other DNA
ctcccactcgttgcacgggcttggcttcgagctcggtaccctcgaggtcattcata

SEQ ID NO: 85 - DNA, 55 bp, synthetic construct
  source 1..55: mol_type = other DNA
atgtctgtcccccccctcgagctcggtaccctcgaggtcattcatatgcttgaga

SEQ ID NO: 86 - DNA, 57 bp, synthetic construct
  source 1..57: mol_type = other DNA
ctccccactcgtttttccgaaggtaaccgagctcggtacccttcgaggtcattcata

SEQ ID NO: 87 - DNA, 42 bp, synthetic construct
  source 1..42: mol_type = other DNA
ctccccactgcttggccctccctgccattcatatgcttgaga

SEQ ID NO: 88 - DNA, 124 bp, synthetic construct
  source 1..124: mol_type = other DNA
acggcatggacgagctgtacaagtaattttttttaccgttcgtatagcatacattatacgaacggtaagccccacgcgcctgtcgcggctccaggagaaggaggagctgcgcgagctcaatgac

SEQ ID NO: 89 - DNA, 121 bp, synthetic construct
  source 1..121: mol_type = other DNA
cccggtgaacagctcctcgcccttgctcaccatataacttcgtataatgtatgctatacgaagttatcgggcggcggagacagcggggcggcgaggccgcgagcgggaccgtgataaggag

SEQ ID NO: 90 - DNA, 20 bp, synthetic construct
  source 1..20: mol_type = other DNA
gtccactccccactcgtgca

SEQ ID NO: 91 - DNA, 42 bp, synthetic construct
  source 1..42: mol_type = other DNA
accgttcgtataatgtatgctatacgaagttatacgagtggg

SEQ ID NO: 92 - DNA, 20 bp, synthetic construct
  source 1..20: mol_type = other DNA
ctctcctacaaacacagggt

SEQ ID NO: 93 - DNA, 41 bp, synthetic construct
  source 1..41: mol_type = other DNA
cttcgtatagcatacattatacgaacggtactgtgtttgta

SEQ ID NO: 94 - DNA, 20 bp, synthetic construct
  source 1..20: mol_type = other DNA
taggagagaaagaatatagc

SEQ ID NO: 95 - DNA, 45 bp, synthetic construct
  source 1..45: mol_type = other DNA
accgttcgtataatgtatgctatacgaagttatatattctttctc

SEQ ID NO: 96 - DNA, 20 bp, synthetic construct
  source 1..20: mol_type = other DNA
aaccaaacgcagacaggaca

SEQ ID NO: 97 - DNA, 39 bp, synthetic construct
  source 1..39: mol_type = other DNA
cttcgtatagcatacattatacgaacggtacctgtctgc

SEQ ID NO: 98 - DNA, 20 bp, synthetic construct
  source 1..20: mol_type = other DNA
tgagaaggagcaagcgagac

SEQ ID NO: 99 - DNA, 39 bp, synthetic construct
  source 1..39: mol_type = other DNA
cttcgtatagcatacattatacgaacggtatcgcttgct

SEQ ID NO: 100 - DNA, 20 bp, synthetic construct
  source 1..20: mol_type = other DNA
atgctagatccgtccctaga

SEQ ID NO: 101 - DNA, 46 bp, synthetic construct
  source 1..46: mol_type = other DNA
accgttcgtataatgtatgctatacgaagttatatatagggacgga

SEQ ID NO: 102 - DNA, 20 bp, synthetic construct
  source 1..20: mol_type = other DNA
ccatgcatgatgcatgggat

SEQ ID NO: 103 - DNA, 40 bp, synthetic construct
  source 1..40: mol_type = other DNA
cttcgtatagcatacattatacgaacggtaccatgcatca